European Patent Application EP 4 198 052 A1, published June 21, 2023. Title: Peptides and antigen binding proteins for use in immunotherapy against fibrolamellar hepatocellular carcinoma (FL-HCC) and other cancers. Applicant: Eberhard Karls Universität Tübingen, Medizinische Fakultät Albert-Ludwigs-Universität. The sequence listing filed with the application follows.

SEQUENCE LISTING (128 sequences)

SEQ ID NO: 1 - protein, 22 aa, artificial sequence
  none
KREIFDRYGEEVKEFLAKAKED

SEQ ID NO: 2 - protein, 16 aa, artificial sequence
  none
EVKEFLAKAKEDFLKK

SEQ ID NO: 3 - protein, 10 aa, artificial sequence
  none
EIFDRYGEEV

SEQ ID NO: 4 - protein, 9 aa, artificial sequence
  none
IFDRYGEEV

SEQ ID NO: 5 - protein, 9 aa, artificial sequence
  none
RYGEEVKEF

SEQ ID NO: 6 - protein, 13 aa, artificial sequence
  none
CAVRDFGNEKLTF

SEQ ID NO: 7 - protein, 14 aa, artificial sequence
  none
CAASRNTGFQKLVF

SEQ ID NO: 8 - protein, 13 aa, artificial sequence
  none
CAVLNFGNEKLTF

SEQ ID NO: 9 - protein, 14 aa, artificial sequence
  none
CAASRKTGANNLFF

SEQ ID NO: 10 - protein, 13 aa, artificial sequence
  none
CAERFSGSEKLVF

SEQ ID NO: 11 - protein, 15 aa, artificial sequence
  none
CAGDRTGGGADGLTF

SEQ ID NO: 12 - protein, 14 aa, artificial sequence
  none
CAASANTGFQKLVF

SEQ ID NO: 13 - protein, 16 aa, artificial sequence
  none
CILRDISNFGNEKLTF

SEQ ID NO: 14 - protein, 13 aa, artificial sequence
  none
CAVLTGGSYIPTF

SEQ ID NO: 15 - protein, 14 aa, artificial sequence
  none
CVVNKAGNNRKLIW

SEQ ID NO: 16 - protein, 14 aa, artificial sequence
  none
CVVNKAGNNRKLIW

SEQ ID NO: 17 - protein, 14 aa, artificial sequence
  none
CIQRRSSNTGKLIF

SEQ ID NO: 18 - protein, 14 aa, artificial sequence
  none
CIQRRSSNTGKLIF

SEQ ID NO: 19 - protein, 12 aa, artificial sequence
  none
CAAQRRSDKLIF

SEQ ID NO: 20 - protein, 12 aa, artificial sequence
  none
CAAQRRSDKLIF

SEQ ID NO: 21 - protein, 12 aa, artificial sequence
  none
CAAQRRSDKLIF

SEQ ID NO: 22 - protein, 16 aa, artificial sequence
  none
CAGRIPTTSGTYKYIF

SEQ ID NO: 23 - protein, 14 aa, artificial sequence
  none
CAVRVLAGGFKTIF

SEQ ID NO: 24 - protein, 11 aa, artificial sequence
  none
CAMKGFQKLVF

SEQ ID NO: 25 - protein, 13 aa, artificial sequence
  none
CALTNFGNEKLTF

SEQ ID NO: 26 - protein, 12 aa, artificial sequence
  none
CAVKGFGNVLHC

SEQ ID NO: 27 - protein, 15 aa, artificial sequence
  none
CALRQYPAAGNKLTF

SEQ ID NO: 28 - protein, 15 aa, artificial sequence
  none
CALRQYPAAGNKLTF

SEQ ID NO: 29 - protein, 15 aa, artificial sequence
  none
CALRQYPASGNKLTF

SEQ ID NO: 30 - protein, 16 aa, artificial sequence
  none
CATPHYSGAGSYQLTF

SEQ ID NO: 31 - protein, 16 aa, artificial sequence
  none
CAVARWVTSGTYKYIF

SEQ ID NO: 32 - protein, 14 aa, artificial sequence
  none
CIQRRSSNTGKLIF

SEQ ID NO: 33 - protein, 14 aa, artificial sequence
  none
CVVNKAGNNRKLIW

SEQ ID NO: 34 - protein, 12 aa, artificial sequence
  none
CAVKGFGNVLHC

SEQ ID NO: 35 - protein, 13 aa, artificial sequence
  none
CALTNFGNEKLTF

SEQ ID NO: 36 - protein, 14 aa, artificial sequence
  none
CASSPLSGGDTQYF

SEQ ID NO: 37 - protein, 14 aa, artificial sequence
  none
CATSRDIVYNEQFF

SEQ ID NO: 38 - protein, 14 aa, artificial sequence
  none
CASSLVTFSYEQYF

SEQ ID NO: 39 - protein, 14 aa, artificial sequence
  none
CASSFGIVRTEAFF

SEQ ID NO: 40 - protein, 15 aa, artificial sequence
  none
CASSPLSGSANEQYF

SEQ ID NO: 41 - protein, 14 aa, artificial sequence
  none
CASTLALGANVLTF

SEQ ID NO: 42 - protein, 16 aa, artificial sequence
  none
CATSRDIVQGANEQFF

SEQ ID NO: 43 - protein, 16 aa, artificial sequence
  none
CATARRRGGREETQYF

SEQ ID NO: 44 - protein, 15 aa, artificial sequence
  none
CASSSYLGPQETQYF

SEQ ID NO: 45 - protein, 14 aa, artificial sequence
  none
CSARDNGRQGEQFF

SEQ ID NO: 46 - protein, 14 aa, artificial sequence
  none
CSARDNGRQGEQFF

SEQ ID NO: 47 - protein, 14 aa, artificial sequence
  none
CSARDNGRQGEQFF

SEQ ID NO: 48 - protein, 14 aa, artificial sequence
  none
CSARDNGRQGEQFF

SEQ ID NO: 49 - protein, 13 aa, artificial sequence
  none
CASSLDLSEKLFF

SEQ ID NO: 50 - protein, 13 aa, artificial sequence
  none
CASSLDLSEKLFF

SEQ ID NO: 51 - protein, 17 aa, artificial sequence
  none
CASSAQSGTGISYEQYF

SEQ ID NO: 52 - protein, 17 aa, artificial sequence
  none
CASSAQSGTGISYEQYF

SEQ ID NO: 53 - protein, 15 aa, artificial sequence
  none
CASSQDLAGGWGYTF

SEQ ID NO: 54 - protein, 15 aa, artificial sequence
  none
CASSQDVGSYTEAFF

SEQ ID NO: 55 - protein, 14 aa, artificial sequence
  none
CASSQAIYTDTQYF

SEQ ID NO: 56 - protein, 14 aa, artificial sequence
  none
CASSQAIYTDTQYF

SEQ ID NO: 57 - protein, 13 aa, artificial sequence
  none
CASSLDLQETQYF

SEQ ID NO: 58 - protein, 13 aa, artificial sequence
  none
CASSLDLQETQYF

SEQ ID NO: 59 - protein, 13 aa, artificial sequence
  none
CASSLDLQETQYF

SEQ ID NO: 60 - protein, 15 aa, artificial sequence
  none
CSARHRDGYSYEQYF

SEQ ID NO: 61 - protein, 14 aa, artificial sequence
  none
CASSSDRATYEQYF

SEQ ID NO: 62 - protein, 17 aa, artificial sequence
  none
CASSAQSGTGISYEQYF

SEQ ID NO: 63 - protein, 13 aa, artificial sequence
  none
CASSLDLSEKLFF

SEQ ID NO: 64 - DNA, 39 bp, artificial sequence
  none
tgtgctgtcagagactttggaaatgagaaattaaccttt

SEQ ID NO: 65 - DNA, 42 bp, artificial sequence
  none
tgtgcagcaagccggaacacaggctttcagaaacttgtattt

SEQ ID NO: 66 - DNA, 39 bp, artificial sequence
  none
tgtgctgttttgaactttggaaatgagaaattaaccttt

SEQ ID NO: 67 - DNA, 42 bp, artificial sequence
  none
tgtgcagcaagccggaaaactggggcaaacaacctcttcttt

SEQ ID NO: 68 - DNA, 39 bp, artificial sequence
  none
tgtgcagagaggtttagcggatctgaaaagctggtcttt

SEQ ID NO: 69 - DNA, 45 bp, artificial sequence
  none
tgtgcaggagacaggacaggaggaggtgctgacggactcaccttt

SEQ ID NO: 70 - DNA, 42 bp, artificial sequence
  none
tgtgcagcaagcgcgaacacaggctttcagaaacttgtattt

SEQ ID NO: 71 - DNA, 48 bp, artificial sequence
  none
tgcatcctgagggatatatctaactttggaaatgagaaattaaccttt

SEQ ID NO: 72 - DNA, 39 bp, artificial sequence
  none
tgtgccgttttaacgggaggaagctacatacctacattt

SEQ ID NO: 73 - DNA, 42 bp, artificial sequence
  none
tgtgtggtgaacaaggctggcaacaaccgtaagctgatttgg

SEQ ID NO: 74 - DNA, 42 bp, artificial sequence; identical to SEQ ID NO: 73
  none

SEQ ID NO: 75 - DNA, 42 bp, artificial sequence
  none
tgcatccaaaggaggtctagcaacacaggcaaactaatcttt

SEQ ID NO: 76 - DNA, 42 bp, artificial sequence; identical to SEQ ID NO: 75
  none

SEQ ID NO: 77 - DNA, 36 bp, artificial sequence
  none
tgtgctgcccaaaggaggagcgacaagctcatcttt

SEQ ID NO: 78 - DNA, 36 bp, artificial sequence; identical to SEQ ID NO: 77
  none

SEQ ID NO: 79 - DNA, 36 bp, artificial sequence; identical to SEQ ID NO: 77
  none

SEQ ID NO: 80 - DNA, 48 bp, artificial sequence
  none
tgtgctgggcggatacctactacctcaggaacctacaaatacatcttt

SEQ ID NO: 81 - DNA, 42 bp, artificial sequence
  none
tgtgctgtgagagtcttggctggaggcttcaaaactatcttt

SEQ ID NO: 82 - DNA, 33 bp, artificial sequence
  none
tgtgcaatgaaaggctttcagaaacttgtattt

SEQ ID NO: 83 - DNA, 39 bp, artificial sequence
  none
tgtgctctgactaactttggaaatgagaaattaaccttt

SEQ ID NO: 84 - DNA, 36 bp, artificial sequence
  none
tgtgctgtgaaaggctttgggaatgtgctgcattgc

SEQ ID NO: 85 - DNA, 45 bp, artificial sequence
  none
tgtgctctgagacagtacccagctgcaggcaacaagctaactttt

SEQ ID NO: 86 - DNA, 45 bp, artificial sequence
  none
tgtgctttgagacagtacccagctgcaggcaacaagctaactttt

SEQ ID NO: 87 - DNA, 45 bp, artificial sequence
  none
tgtgctctgagacagtacccagcttcaggcaacaagctaactttt

SEQ ID NO: 88 - DNA, 48 bp, artificial sequence
  none
tgtgctacgcctcattactctggggctgggagttaccaactcactttc

SEQ ID NO: 89 - DNA, 48 bp, artificial sequence
  none
tgtgccgtggcccgatgggtaacctcaggaacctacaaatacatcttt

SEQ ID NO: 90 - DNA, 42 bp, artificial sequence; identical to SEQ ID NO: 75
  none

SEQ ID NO: 91 - DNA, 42 bp, artificial sequence; identical to SEQ ID NO: 73
  none

SEQ ID NO: 92 - DNA, 36 bp, artificial sequence; identical to SEQ ID NO: 84
  none

SEQ ID NO: 93 - DNA, 39 bp, artificial sequence; identical to SEQ ID NO: 83
  none

SEQ ID NO: 94 - DNA, 42 bp, artificial sequence
  none
tgtgccagctcaccactatcggggggagatacgcagtatttt

SEQ ID NO: 95 - DNA, 42 bp, artificial sequence
  none
tgtgccaccagcagagatatagtatacaatgagcagttcttc

SEQ ID NO: 96 - DNA, 42 bp, artificial sequence
  none
tgtgccagcagcttagttacgttctcctacgagcagtacttc

SEQ ID NO: 97 - DNA, 42 bp, artificial sequence
  none
tgtgccagcagcttcgggatagtcaggactgaagctttcttt

SEQ ID NO: 98 - DNA, 45 bp, artificial sequence
  none
tgtgccagctcaccactgagcgggagtgccaacgagcagtacttc

SEQ ID NO: 99 - DNA, 42 bp, artificial sequence
  none
tgtgccagcaccctggccctcggggccaacgtcctgactttc

SEQ ID NO: 100 - DNA, 48 bp, artificial sequence
  none
tgtgccaccagcagagatatcgttcagggggcaaatgagcagttcttc

SEQ ID NO: 101 - DNA, 48 bp, artificial sequence
  none
tgtgccaccgcacgccgtcggggggggcgggaagagacccagtacttc

SEQ ID NO: 102 - DNA, 45 bp, artificial sequence
  none
tgtgccagcagctcttacctagggccacaagagacccagtacttc

SEQ ID NO: 103 - DNA, 42 bp, artificial sequence
  none
tgcagtgctagagataacggacgtcagggtgagcagttcttc

SEQ ID NO: 104 - DNA, 42 bp, artificial sequence; identical to SEQ ID NO: 103
  none

SEQ ID NO: 105 - DNA, 42 bp, artificial sequence; identical to SEQ ID NO: 103
  none

SEQ ID NO: 106 - DNA, 42 bp, artificial sequence; identical to SEQ ID NO: 103
  none

SEQ ID NO: 107 - DNA, 39 bp, artificial sequence
  none
tgtgctagcagcttagacttgtcggaaaaactgtttttt

SEQ ID NO: 108 - DNA, 39 bp, artificial sequence; identical to SEQ ID NO: 107
  none

SEQ ID NO: 109 - DNA, 51 bp, artificial sequence
  none
tgcgccagcagcgcgcaatctgggacagggatctcctacgagcagtacttc

SEQ ID NO: 110 - DNA, 51 bp, artificial sequence; identical to SEQ ID NO: 109
  none

SEQ ID NO: 111 - DNA, 45 bp, artificial sequence
  none
tgcgccagcagccaagatctggcagggggctggggctacaccttc

SEQ ID NO: 112 - DNA, 45 bp, artificial sequence
  none
tgcgccagcagccaagacgtcggcagctacactgaagctttcttt

SEQ ID NO: 113 - DNA, 42 bp, artificial sequence
  none
tgcgccagcagccaagccatttatacagatacgcagtatttt

SEQ ID NO: 114 - DNA, 42 bp, artificial sequence; identical to SEQ ID NO: 113
  none

SEQ ID NO: 115 - DNA, 39 bp, artificial sequence
  none
tgtgccagcagcttggacctccaagagacccagtacttc

SEQ ID NO: 116 - DNA, 39 bp, artificial sequence; identical to SEQ ID NO: 115
  none

SEQ ID NO: 117 - DNA, 39 bp, artificial sequence; identical to SEQ ID NO: 115
  none

SEQ ID NO: 118 - DNA, 45 bp, artificial sequence
  none
tgcagtgctagacatcgggacggttacagttacgagcagtacttc

SEQ ID NO: 119 - DNA, 42 bp, artificial sequence
  none
tgtgccagcagctcggacagggcgacctacgagcagtacttc

SEQ ID NO: 120 - DNA, 51 bp, artificial sequence; identical to SEQ ID NO: 109
  none

SEQ ID NO: 121 - DNA, 39 bp, artificial sequence; identical to SEQ ID NO: 107
  none

SEQ ID NO: 122 - DNA, 20 bp, artificial sequence
  primer
gttcaaggagatcgctgagg

SEQ ID NO: 123 - DNA, 20 bp, artificial sequence
  primer
ttcccggtctccttgtgttt

SEQ ID NO: 124 - protein, 9 aa, artificial sequence
  none
YLLPAIVHI

SEQ ID NO: 125 - protein, 15 aa, artificial sequence
  none
ETVITVDTKAAGKGK

SEQ ID NO: 126 - protein, 9 aa, artificial sequence
  none
KYPENFFLL

SEQ ID NO: 127 - protein, 9 aa, artificial sequence
  none
EEFGRAFSF

SEQ ID NO: 128 - protein, 9 aa, artificial sequence
  none
TYSEKTTLF